European Patent Application EP 4 410 816 A1, published August 7, 2024. Title: Peptide. Applicant: PeptiDream Inc. The sequence listing filed with the application follows.

SEQUENCE LISTING (70 sequences)

SEQ ID NO: 1 - protein, 16 aa, synthetic construct
  REGION 1..16: note = artificial peptide
  MUTAGEN 2: note = X stands for an amino acid having a side chain of unsubstitutedor substituted aromatic ring
  MUTAGEN 4: note = X stands for any amino acid
  MUTAGEN 7: note = X stands for any amino acid
  MUTAGEN 8: note = X stands for any amino acid
  MUTAGEN 9: note = X stands for any amino acid
  MUTAGEN 10: note = X stands for an amino acid having a side chain of unsubstitutedor substituted alkyl, or a secondary amino acid havingunsubstituted or substituted alkyl
  MUTAGEN 12: note = X stands for an amino acid having a side chain of unsubstitutedor substituted aromatic ring
  MUTAGEN 13: note = X stands for an amino acid having a side chain of unsubstitutedor substituted aromatic ring
  MUTAGEN 14: note = X stands for any amino acid
  MUTAGEN 15: note = X stands for any amino acid
FXVXNVXXXXVXXXXC

SEQ ID NO: 2 - protein, 17 aa, synthetic construct
  REGION 1..17: note = artificial peptide
  MUTAGEN 2: note = X stands for 1-naphthyl-L-alanine
  MUTAGEN 10: note = X stands for phenethylglycine
  MUTAGEN 12: note = X stands for 1-naphthyl-L-alanine
FXVVNVYDDXVXYHVCG

SEQ ID NO: 3 - protein, 16 aa, synthetic construct
  REGION 1..16: note = artificial peptide
  MUTAGEN 2: note = X stands for 1-naphthyl-L-alanine
  MUTAGEN 10: note = X stands for phenethylglycine
  MUTAGEN 12: note = X stands for 1-naphthyl-L-alanine
FXVVNVYDDXVXYHVC

SEQ ID NO: 4 - protein, 17 aa, synthetic construct
  REGION 1..17: note = artificial peptide
  MUTAGEN 10: note = X stands for phenethylglycine
  MUTAGEN 12: note = X stands for 1-naphthyl-L-alanine
FWVVNVYDDXVXYHVCG

SEQ ID NO: 5 - protein, 17 aa, synthetic construct
  REGION 1..17: note = artificial peptide
  MUTAGEN 2: note = X stands for 6-aza-L-tryptophan
  MUTAGEN 10: note = X stands for phenethylglycine
  MUTAGEN 12: note = X stands for 1-naphthyl-L-alanine
FXVVNVYDDXVXYHVCG

SEQ ID NO: 6 - protein, 17 aa, synthetic construct
  REGION 1..17: note = artificial peptide
  MUTAGEN 2: note = X stands for L-7-azatryptophan
  MUTAGEN 10: note = X stands for phenethylglycine
  MUTAGEN 12: note = X stands for 1-naphthyl-L-alanine
FXVVNVYDDXVXYHVCG

SEQ ID NO: 7 - protein, 17 aa, synthetic construct
  REGION 1..17: note = artificial peptide
  MUTAGEN 2: note = X stands for 1-naphthyl-L-alanine
  MUTAGEN 7: note = X stands for 4-pyridyl-L-alanine
  MUTAGEN 10: note = X stands for phenethylglycine
  MUTAGEN 12: note = X stands for 1-naphthyl-L-alanine
FXVVNVXDDXVXYHVCG

SEQ ID NO: 8 - protein, 17 aa, synthetic construct
  REGION 1..17: note = artificial peptide
  MUTAGEN 2: note = X stands for 1-naphthyl-L-alanine
  MUTAGEN 7: note = X stands for 4-pyridyl-L-alanine
  MUTAGEN 10: note = X stands for phenethylglycine
  MUTAGEN 12: note = X stands for 1-naphthyl-L-alanine
FXVKNVXDDXVXYHVCG

SEQ ID NO: 9 - protein, 17 aa, synthetic construct
  REGION 1..17: note = artificial peptide
  MUTAGEN 2: note = X stands for L-7-azatryptophan
  MUTAGEN 7: note = X stands for 4-pyridyl-L-alanine
  MUTAGEN 10: note = X stands for phenethylglycine
  MUTAGEN 12: note = X stands for 1-naphthyl-L-alanine
FXVVNVXDDXVXYHVCG

SEQ ID NO: 10 - protein, 17 aa, synthetic construct
  REGION 1..17: note = artificial peptide
  MUTAGEN 2: note = X stands for 1-naphthyl-L-alanine
  MUTAGEN 7: note = X stands for 4-pyridyl-L-alanine
  MUTAGEN 10: note = X stands for phenethylglycine
  MUTAGEN 12: note = X stands for 1-naphthyl-L-alanine
  MUTAGEN 13: note = X stands for 4-pyridyl-L-alanine
FXVVNVXDDXVXXHVCG

SEQ ID NO: 11 - protein, 17 aa, synthetic construct
  REGION 1..17: note = artificial peptide
  MUTAGEN 2: note = X stands for 1-naphthyl-L-alanine
  MUTAGEN 4: note = X stands for N6-(4-(carboxymethyl)piperazine-1-carbonyl)-L-lysine
  MUTAGEN 7: note = X stands for 4-pyridyl-L-alanine
  MUTAGEN 10: note = X stands for phenethylglycine
  MUTAGEN 12: note = X stands for 1-naphthyl-L-alanine
FXVXNVXDDXVXYHVCG

SEQ ID NO: 12 - protein, 17 aa, synthetic construct
  REGION 1..17: note = artificial peptide
  MUTAGEN 2: note = X stands for 1-naphthyl-L-alanine
  MUTAGEN 7: note = X stands for 4-pyridyl-L-alanine
  MUTAGEN 9: note = X stands for N6-(4-(carboxymethyl)piperazine-1-carbonyl)-L-lysine
  MUTAGEN 10: note = X stands for phenethylglycine
  MUTAGEN 12: note = X stands for 1-naphthyl-L-alanine
FXVVNVXDXXVXYHVCG

SEQ ID NO: 13 - protein, 17 aa, synthetic construct
  REGION 1..17: note = artificial peptide
  MUTAGEN 2: note = X stands for 1-naphthyl-L-alanine
  MUTAGEN 7: note = X stands for 4-pyridyl-L-alanine
  MUTAGEN 10: note = X stands for phenethylglycine
  MUTAGEN 12: note = X stands for 1-naphthyl-L-alanine
  MUTAGEN 15: note = X stands for N6-(4-(carboxymethyl)piperazine-1-carbonyl)-L-lysine
FXVVNVXDDXVXYHXCG

SEQ ID NO: 14 - protein, 16 aa, synthetic construct
  REGION 1..16: note = artificial peptide
  MUTAGEN 2: note = X stands for 1-naphthyl-L-alanine
  MUTAGEN 7: note = X stands for 4-pyridyl-L-alanine
  MUTAGEN 10: note = X stands for phenethylglycine
  MUTAGEN 12: note = X stands for 1-naphthyl-L-alanine
  MUTAGEN 15: note = X stands for N6-(4-(carboxymethyl)piperazine-1-carbonyl)-L-lysine
FXVVNVXDDXVXYHXC

SEQ ID NO: 15 - protein, 17 aa, synthetic construct
  REGION 1..17: note = artificial peptide
  MUTAGEN 2: note = X stands for 1-naphthyl-L-alanine
  MUTAGEN 4: note = X stands for N6-(methyl-((2S,3R,4R,5R)-2,3,4,5,6-pentahydroxyhexyl)carbamoyl)-L-lysine
  MUTAGEN 7: note = X stands for 4-pyridyl-L-alanine
  MUTAGEN 10: note = X stands for phenethylglycine
  MUTAGEN 12: note = X stands for 1-naphthyl-L-alanine
FXVXNVXDDXVXYHVCG

SEQ ID NO: 16 - protein, 17 aa, synthetic construct
  REGION 1..17: note = artificial peptide
  MUTAGEN 2: note = X stands for 1-naphthyl-L-alanine
  MUTAGEN 7: note = X stands for 4-pyridyl-L-alanine
  MUTAGEN 9: note = X stands for N6-(methyl-((2S,3R,4R,5R)-2,3,4,5,6-pentahydroxyhexyl)carbamoyl)-L-lysine
  MUTAGEN 10: note = X stands for phenethylglycine
  MUTAGEN 12: note = X stands for 1-naphthyl-L-alanine
FXVVNVXDXXVXYHVCG

SEQ ID NO: 17 - protein, 17 aa, synthetic construct
  REGION 1..17: note = artificial peptide
  MUTAGEN 2: note = X stands for 1-naphthyl-L-alanine
  MUTAGEN 7: note = X stands for 4-pyridyl-L-alanine
  MUTAGEN 10: note = X stands for phenethylglycine
  MUTAGEN 12: note = X stands for 1-naphthyl-L-alanine
  MUTAGEN 15: note = X stands for N6-(methyl-((2S,3R,4R,5R)-2,3,4,5,6-pentahydroxyhexyl)carbamoyl)-L-lysine
FXVVNVXDDXVXYHXCG

SEQ ID NO: 18 - protein, 17 aa, synthetic construct
  REGION 1..17: note = artificial peptide
  MUTAGEN 2: note = X stands for L-7-azatryptophan
  MUTAGEN 7: note = X stands for 4-pyridyl-L-alanine
  MUTAGEN 9: note = X stands for N6-(4-(carboxymethyl)piperazine-1-carbonyl)-L-lysine
  MUTAGEN 10: note = X stands for phenethylglycine
  MUTAGEN 12: note = X stands for 1-naphthyl-L-alanine
FXVVNVXDXXVXYHVCG

SEQ ID NO: 19 - protein, 17 aa, synthetic construct
  REGION 1..17: note = artificial peptide
  MUTAGEN 2: note = X stands for L-7-azatryptophan
  MUTAGEN 7: note = X stands for 4-pyridyl-L-alanine
  MUTAGEN 9: note = X stands for N6-(methyl-((2S,3R,4R,5R)-2,3,4,5,6-pentahydroxyhexyl)carbamoyl)-L-lysine
  MUTAGEN 10: note = X stands for phenethylglycine
  MUTAGEN 12: note = X stands for 1-naphthyl-L-alanine
FXVVNVXDXXVXYHVCG

SEQ ID NO: 20 - protein, 17 aa, synthetic construct
  REGION 1..17: note = artificial peptide
  MUTAGEN 2: note = X stands for 1-naphthyl-L-alanine
  MUTAGEN 4: note = X stands for N6-(4-(carboxymethyl)piperazine-1-carbonyl)-L-lysine
  MUTAGEN 7: note = X stands for 4-pyridyl-L-alanine
  MUTAGEN 10: note = X stands for phenethylglycine
  MUTAGEN 12: note = X stands for 1-naphthyl-L-alanine
  MUTAGEN 15: note = X stands for N6-(4-(carboxymethyl)piperazine-1-carbonyl)-L-lysine
FXVXNVXDDXVXYHXCG

SEQ ID NO: 21 - protein, 17 aa, synthetic construct
  REGION 1..17: note = artificial peptide
  MUTAGEN 2: note = X stands for 1-naphthyl-L-alanine
  MUTAGEN 4: note = X stands for N6-(methyl-((2S,3R,4R,5R)-2,3,4,5,6-pentahydroxyhexyl)carbamoyl)-L-lysine
  MUTAGEN 7: note = X stands for 4-pyridyl-L-alanine
  MUTAGEN 10: note = X stands for phenethylglycine
  MUTAGEN 12: note = X stands for 1-naphthyl-L-alanine
  MUTAGEN 15: note = X stands for N6-(4-(carboxymethyl)piperazine-1-carbonyl)-L-lysine
FXVXNVXDDXVXYHXCG

SEQ ID NO: 22 - protein, 17 aa, synthetic construct
  REGION 1..17: note = artificial peptide
  MUTAGEN 2: note = X stands for 1-naphthyl-L-alanine
  MUTAGEN 7: note = X stands for 4-pyridyl-L-alanine
  MUTAGEN 10: note = X stands for phenethylglycine
  MUTAGEN 12: note = X stands for 1-naphthyl-L-alanine
  MUTAGEN 15: note = X stands for N6-(4-(carboxymethyl)piperazine-1-carbonyl)-L-lysine
FXVVNVXDEXVXYHXCG

SEQ ID NO: 23 - protein, 17 aa, synthetic construct
  REGION 1..17: note = artificial peptide
  MUTAGEN 2: note = X stands for 1-naphthyl-L-alanine
  MUTAGEN 7: note = X stands for 4-pyridyl-L-alanine
  MUTAGEN 9: note = X stands for N6-(4-(carboxymethyl)piperazine-1-carbonyl)-L-lysine
  MUTAGEN 10: note = X stands for phenethylglycine
  MUTAGEN 12: note = X stands for 1-naphthyl-L-alanine
  MUTAGEN 15: note = X stands for N6-(4-(carboxymethyl)piperazine-1-carbonyl)-L-lysine
FXVVNVXDXXVXYHXCG

SEQ ID NO: 24 - protein, 17 aa, synthetic construct
  REGION 1..17: note = artificial peptide
  MUTAGEN 2: note = X stands for 1-naphthyl-L-alanine
  MUTAGEN 7: note = X stands for 4-pyridyl-L-alanine
  MUTAGEN 9: note = X stands for N6-(methyl-((2S,3R,4R,5R)-2,3,4,5,6-pentahydroxyhexyl)carbamoyl)-L-lysine
  MUTAGEN 10: note = X stands for phenethylglycine
  MUTAGEN 12: note = X stands for 1-naphthyl-L-alanine
  MUTAGEN 15: note = X stands for N6-(4-(carboxymethyl)piperazine-1-carbonyl)-L-lysine
FXVVNVXDXXVXYHXCG

SEQ ID NO: 25 - protein, 17 aa, synthetic construct
  REGION 1..17: note = artificial peptide
  MUTAGEN 2: note = X stands for 1-naphthyl-L-alanine
  MUTAGEN 4: note = X stands for N6-(methyl-((2S,3R,4R,5R)-2,3,4,5,6-pentahydroxyhexyl)carbamoyl)-L-lysine
  MUTAGEN 7: note = X stands for 4-pyridyl-L-alanine
  MUTAGEN 10: note = X stands for phenethylglycine
  MUTAGEN 12: note = X stands for 1-naphthyl-L-alanine
  MUTAGEN 15: note = X stands for N6-(4-(carboxymethyl)piperazine-1-carbonyl)-L-lysine
FXVXNVXDEXVXYHXCG

SEQ ID NO: 26 - protein, 17 aa, synthetic construct
  REGION 1..17: note = artificial peptide
  MUTAGEN 2: note = X stands for 1-naphthyl-L-alanine
  MUTAGEN 4: note = X stands for N6-(methyl-((2S,3R,4R,5R)-2,3,4,5,6-pentahydroxyhexyl)carbamoyl)-L-lysine
  MUTAGEN 7: note = X stands for 4-pyridyl-L-alanine
  MUTAGEN 9: note = X stands for N6-(4-(carboxymethyl)piperazine-1-carbonyl)-L-lysine
  MUTAGEN 10: note = X stands for phenethylglycine
  MUTAGEN 12: note = X stands for 1-naphthyl-L-alanine
  MUTAGEN 15: note = X stands for N6-(4-(carboxymethyl)piperazine-1-carbonyl)-L-lysine
FXVXNVXDXXVXYHXCG

SEQ ID NO: 27 - protein, 17 aa, synthetic construct
  REGION 1..17: note = artificial peptide
  MUTAGEN 2: note = X stands for 1-naphthyl-L-alanine
  MUTAGEN 4: note = X stands for N6-(methyl-((2S,3R,4R,5R)-2,3,4,5,6-pentahydroxyhexyl)carbamoyl)-L-lysine
  MUTAGEN 7: note = X stands for 4-pyridyl-L-alanine
  MUTAGEN 9: note = X stands for N6-(methyl-((2S,3R,4R,5R)-2,3,4,5,6-pentahydroxyhexyl)carbamoyl)-L-lysine
  MUTAGEN 10: note = X stands for phenethylglycine
  MUTAGEN 12: note = X stands for 1-naphthyl-L-alanine
  MUTAGEN 15: note = X stands for N6-(4-(carboxymethyl)piperazine-1-carbonyl)-L-lysine
FXVXNVXDXXVXYHXCG

SEQ ID NO: 28 - protein, 17 aa, synthetic construct
  REGION 1..17: note = artificial peptide
  MUTAGEN 2: note = X stands for 1-naphthyl-L-alanine
  MUTAGEN 7: note = X stands for 4-pyridyl-L-alanine
  MUTAGEN 10: note = X stands for phenethylglycine
  MUTAGEN 12: note = X stands for 1-naphthyl-L-alanine
FXVVNVXDDXVXYHECG

SEQ ID NO: 29 - protein, 17 aa, synthetic construct
  REGION 1..17: note = artificial peptide
  MUTAGEN 2: note = X stands for 1-naphthyl-L-alanine
  MUTAGEN 4: note = X stands for N6-(methyl-((2S,3R,4R,5R)-2,3,4,5,6-pentahydroxyhexyl)carbamoyl)-L-lysine
  MUTAGEN 7: note = X stands for 4-pyridyl-L-alanine
  MUTAGEN 10: note = X stands for phenethylglycine
  MUTAGEN 12: note = X stands for 1-naphthyl-L-alanine
FXVXNVXDDXVXYHECG

SEQ ID NO: 30 - protein, 17 aa, synthetic construct
  REGION 1..17: note = artificial peptide
  MUTAGEN 2: note = X stands for 1-naphthyl-L-alanine
  MUTAGEN 4: note = X stands for N6-(methyl-((2S,3R,4R,5R)-2,3,4,5,6-pentahydroxyhexyl)carbamoyl)-L-lysine
  MUTAGEN 7: note = X stands for 4-pyridyl-L-alanine
  MUTAGEN 10: note = X stands for phenethylglycine
  MUTAGEN 12: note = X stands for 1-naphthyl-L-alanine
FXVXNVXDEXVXYHECG

SEQ ID NO: 31 - protein, 17 aa, synthetic construct
  REGION 1..17: note = artificial peptide
  MUTAGEN 2: note = X stands for 1-naphthyl-L-alanine
  MUTAGEN 4: note = X stands for N6-(methyl-((2S,3R,4R,5R)-2,3,4,5,6-pentahydroxyhexyl)carbamoyl)-L-lysine
  MUTAGEN 7: note = X stands for 4-pyridyl-L-alanine
  MUTAGEN 9: note = X stands for N6-(methyl-((2S,3R,4R,5R)-2,3,4,5,6-pentahydroxyhexyl)carbamoyl)-L-lysine
  MUTAGEN 10: note = X stands for phenethylglycine
  MUTAGEN 12: note = X stands for 1-naphthyl-L-alanine
FXVXNVXDXXVXYHECG

SEQ ID NO: 32 - protein, 18 aa, synthetic construct
  REGION 1..18: note = artificial peptide
  MUTAGEN 2: note = X stands for 1-naphthyl-L-alanine
  MUTAGEN 7: note = X stands for 4-pyridyl-L-alanine
  MUTAGEN 10: note = X stands for phenethylglycine
  MUTAGEN 12: note = X stands for 1-naphthyl-L-alanine
  MUTAGEN 15: note = X stands for N6-(4-(carboxymethyl)piperazine-1-carbonyl)-L-lysine
  BINDING 18: note = Lys is bounded by 2, 5, 8, 11, 14, 17, 20, 23-octaoxahexacosane-26-oic acid
FXVVNVXDDXVXYHXCGK

SEQ ID NO: 33 - protein, 18 aa, synthetic construct
  REGION 1..18: note = artificial peptide
  MUTAGEN 2: note = X stands for 1-naphthyl-L-alanine
  MUTAGEN 7: note = X stands for 4-pyridyl-L-alanine
  MUTAGEN 10: note = X stands for phenethylglycine
  MUTAGEN 12: note = X stands for 1-naphthyl-L-alanine
  MUTAGEN 15: note = X stands for N6-(4-(carboxymethyl)piperazine-1-carbonyl)-L-lysine
  BINDING 18: note = Lys is bounded by methoxypolyethyleneglycolcarbonate
FXVVNVXDDXVXYHXCGK

SEQ ID NO: 34 - protein, 17 aa, synthetic construct
  REGION 1..17: note = artificial peptide
  MUTAGEN 2: note = X stands for 1-naphthyl-L-alanine
  MUTAGEN 10: note = X stands for phenethylglycine
FXVVNVYDDXVWYHVCG

SEQ ID NO: 35 - protein, 17 aa, synthetic construct
  REGION 1..17: note = artificial peptide
  MUTAGEN 2: note = X stands for 1-naphthyl-L-alanine
  MUTAGEN 10: note = X stands for phenethylglycine
  MUTAGEN 12: note = X stands for 1-naphthyl-L-alanine
FXVVNVYDDXVXEHVCG

SEQ ID NO: 36 - protein, 17 aa, synthetic construct
  REGION 1..17: note = artificial peptide
  MUTAGEN 2: note = X stands for 1-naphthyl-L-alanine
  MUTAGEN 10: note = X stands for phenethylglycine
  MUTAGEN 12: note = X stands for 6-aza-L-tryptophan
FXVVNVYDDXVXYHVCG

SEQ ID NO: 37 - protein, 17 aa, synthetic construct
  REGION 1..17: note = artificial peptide
  MUTAGEN 2: note = X stands for 1-naphthyl-L-alanine
  MUTAGEN 10: note = X stands for phenethylglycine
  MUTAGEN 12: note = X stands for 1-naphthyl-L-alanine
FXVVNVYDDXVXYEVCG

SEQ ID NO: 38 - protein, 17 aa, synthetic construct
  REGION 1..17: note = artificial peptide
  MUTAGEN 2: note = X stands for 1-naphthyl-L-alanine
  MUTAGEN 10: note = X stands for phenethylglycine
  MUTAGEN 12: note = X stands for 1-naphthyl-L-alanine
FXVVNVYADXVXYHVCG

SEQ ID NO: 39 - protein, 17 aa, synthetic construct
  REGION 1..17: note = artificial peptide
  MUTAGEN 2: note = X stands for 1-naphthyl-L-alanine
  MUTAGEN 10: note = X stands for phenethylglycine
  MUTAGEN 12: note = X stands for 1-naphthyl-L-alanine
FXVQNVYDDXVXYHVCG

SEQ ID NO: 40 - protein, 17 aa, synthetic construct
  REGION 1..17: note = artificial peptide
  MUTAGEN 2: note = X stands for 1-naphthyl-L-alanine
  MUTAGEN 10: note = X stands for phenenethylglycine
  MUTAGEN 12: note = X stands for 1-naphthyl-L-alanine
FXVVNVYDDXVXYHACG

SEQ ID NO: 41 - protein, 17 aa, synthetic construct
  REGION 1..17: note = artificial peptide
  MUTAGEN 2: note = X stands for 1-naphthyl-L-alanine
  MUTAGEN 10: note = X stands for methylglycine
  MUTAGEN 12: note = X stands for 1-naphthyl-L-alanine
FXVVNVYDDXVXYHVCG

SEQ ID NO: 42 - protein, 17 aa, synthetic construct
  REGION 1..17: note = artificial peptide
  MUTAGEN 2: note = X stands for 1-naphthyl-L-alanine
  MUTAGEN 10: note = X stands for phenethylglycine
  MUTAGEN 12: note = X stands for 1-naphthyl-L-alanine
FXVVNVYDAXVXYHVCG

SEQ ID NO: 43 - protein, 17 aa, synthetic construct
  REGION 1..17: note = artificial peptide
  MUTAGEN 2: note = X stands for 1-naphthyl-L-alanine
  MUTAGEN 10: note = X stands for phenethylglycine
  MUTAGEN 12: note = X stands for 1-naphthyl-L-alanine
FXVVNVYDDXVXYAVCG

SEQ ID NO: 44 - protein, 17 aa, synthetic construct
  REGION 1..17: note = artificial peptide
  MUTAGEN 2: note = X stands for 1-naphthyl-L-alanine
  MUTAGEN 10: note = X stands for phenethylglycine
  MUTAGEN 12: note = X stands for 1-naphthyl-L-alanine
FXVVNVYDDXVXYHKCG

SEQ ID NO: 45 - protein, 17 aa, synthetic construct
  REGION 1..17: note = artificial peptide
  MUTAGEN 2: note = X stands for 1-naphthyl-L-alanine
  MUTAGEN 10: note = X stands for phenethylglycine
  MUTAGEN 12: note = X stands for 1-naphthyl-L-alanine
FXVVNVYQDXVXYHVCG

SEQ ID NO: 46 - protein, 17 aa, synthetic construct
  REGION 1..17: note = artificial peptide
  MUTAGEN 2: note = X stands for 1-naphthyl-L-alanine
  MUTAGEN 10: note = X stands for phenethylglycine
  MUTAGEN 12: note = X stands for 1-naphthyl-L-alanine
FXVVNVADDXVXYHVCG

SEQ ID NO: 47 - protein, 17 aa, synthetic construct
  REGION 1..17: note = artificial peptide
  MUTAGEN 2: note = X stands for 1-naphthyl-L-alanine
  MUTAGEN 10: note = X stands for phenethylglycine
  MUTAGEN 12: note = X stands for 1-naphthyl-L-alanine
FXVVNVYDDXVXYQVCG

SEQ ID NO: 48 - protein, 17 aa, synthetic construct
  REGION 1..17: note = artificial peptide
  MUTAGEN 2: note = X stands for 1-naphthyl-L-alanine
  MUTAGEN 10: note = X stands for phenethylglycine
  MUTAGEN 12: note = X stands for 1-naphthyl-L-alanine
FXVVNVEDDXVXYHVCG

SEQ ID NO: 49 - protein, 17 aa, synthetic construct
  REGION 1..17: note = artificial peptide
  MUTAGEN 2: note = X stands for 1-naphthyl-L-alanine
  MUTAGEN 10: note = X stands for phenethylglycine
  MUTAGEN 12: note = X stands for 1-naphthyl-L-alanine
  MUTAGEN 13: note = X stands for 4-pyridyl-L-alanine
FXVVNVYDDXVXXHVCG

SEQ ID NO: 50 - protein, 17 aa, synthetic construct
  REGION 1..17: note = artificial peptide
  MUTAGEN 2: note = X stands for 1-naphthyl-L-alanine
  MUTAGEN 10: note = X stands for phenethylglycine
  MUTAGEN 12: note = X stands for 1-naphthyl-L-alanine
FXVVNVYDDXVXYHQCG

SEQ ID NO: 51 - protein, 17 aa, synthetic construct
  REGION 1..17: note = artificial peptide
  MUTAGEN 2: note = X stands for 1-naphthyl-L-alanine
  MUTAGEN 10: note = X stands for phenethylglycine
  MUTAGEN 12: note = X stands for 1-naphthyl-L-alanine
FXVKNVYDDXVXYHVCG

SEQ ID NO: 52 - protein, 17 aa, synthetic construct
  REGION 1..17: note = artificial peptide
  MUTAGEN 2: note = X stands for 6-aza-L-tryptophan
  MUTAGEN 10: note = X stands for phenethylglycine
  MUTAGEN 12: note = X stands for 1-naphthyl-L-alanine
FXVVNVYDDXVXYHVCG

SEQ ID NO: 53 - protein, 17 aa, synthetic construct
  REGION 1..17: note = artificial peptide
  MUTAGEN 2: note = X stands for 1-naphthyl-L-alanine
  MUTAGEN 12: note = X stands for 1-naphthyl-L-alanine
FXVVNVYDDKVXYHVCG

SEQ ID NO: 54 - protein, 17 aa, synthetic construct
  REGION 1..17: note = artificial peptide
  MUTAGEN 2: note = X stands for 1-naphthyl-L-alanine
  MUTAGEN 7: note = X stands for p-guanidino-L-phenylalanine
  MUTAGEN 10: note = X stands for phenethylglycine
  MUTAGEN 12: note = X stands for 1-naphthyl-L-alanine
FXVVNVXDDXVXYHVCG

SEQ ID NO: 55 - protein, 17 aa, synthetic construct
  REGION 1..17: note = artificial peptide
  MUTAGEN 2: note = X stands for 1-naphthyl-L-alanine
  MUTAGEN 10: note = X stands for phenethylglycine
  MUTAGEN 12: note = X stands for 1-naphthyl-L-alanine
FXVVNVYDDXVXYHECG

SEQ ID NO: 56 - protein, 17 aa, synthetic construct
  REGION 1..17: note = artificial peptide
  MUTAGEN 10: note = X stands for phenethylglycine
  MUTAGEN 12: note = X stands for 1-naphthyl-L-alanine
FWVVNVYDDXVXYHVCG

SEQ ID NO: 57 - protein, 17 aa, synthetic construct
  REGION 1..17: note = artificial peptide
  MUTAGEN 2: note = X stands for 1-naphthyl-L-alanine
  MUTAGEN 10: note = X stands for phenethylglycine
  MUTAGEN 12: note = X stands for 1-naphthyl-L-alanine
FXVVNVQDDXVXYHVCG

SEQ ID NO: 58 - protein, 17 aa, synthetic construct
  REGION 1..17: note = artificial peptide
  MUTAGEN 2: note = X stands for 1-naphthyl-L-alanine
  MUTAGEN 10: note = X stands for phenethylglycine
  MUTAGEN 12: note = X stands for 1-naphthyl-L-alanine
FXVVNVYEDXVXYHVCG

SEQ ID NO: 59 - protein, 17 aa, synthetic construct
  REGION 1..17: note = artificial peptide
  MUTAGEN 2: note = X stands for 1-naphthyl-L-alanine
  MUTAGEN 10: note = X stands for phenethylglycine
  MUTAGEN 12: note = X stands for 1-naphthyl-L-alanine
  MUTAGEN 13: note = X stands for 3-(3-pyridyl)-L-alanine
FXVVNVYDDXVXXHVCG

SEQ ID NO: 60 - protein, 17 aa, synthetic construct
  REGION 1..17: note = artificial peptide
  MUTAGEN 2: note = X stands for 1-naphthyl-L-alanine
  MUTAGEN 10: note = X stands for phenethylglycine
  MUTAGEN 12: note = X stands for 1-naphthyl-L-alanine
FXVVNVYDQXVXYHVCG

SEQ ID NO: 61 - protein, 17 aa, synthetic construct
  REGION 1..17: note = artificial peptide
  MUTAGEN 2: note = X stands for 1-naphthyl-L-alanine
  MUTAGEN 10: note = X stands for phenethylglycine
  MUTAGEN 12: note = X stands for 1-naphthyl-L-alanine
FXVVNVYKDXVXYHVCG

SEQ ID NO: 62 - protein, 17 aa, synthetic construct
  REGION 1..17: note = artificial peptide
  MUTAGEN 2: note = X stands for 1-naphthyl-L-alanine
  MUTAGEN 10: note = X stands for phenethylglycine
  MUTAGEN 12: note = X stands for 1-naphthyl-L-alanine
FXVVNVYDDXVXYHVCG

SEQ ID NO: 63 - protein, 17 aa, synthetic construct
  REGION 1..17: note = artificial peptide
  MUTAGEN 2: note = X stands for 1-naphthyl-L-alanine
  MUTAGEN 10: note = X stands for phenethylglycine
  MUTAGEN 12: note = X stands for 1-naphthyl-L-alanine
FXVVNVKDDXVXYHVCG

SEQ ID NO: 64 - protein, 17 aa, synthetic construct
  REGION 1..17: note = artificial peptide
  MUTAGEN 2: note = X stands for 1-naphthyl-L-alanine
  MUTAGEN 10: note = X stands for phenethylglycine
  MUTAGEN 12: note = X stands for 1-naphthyl-L-alanine
FXVVNVYDKXVXYHVCG

SEQ ID NO: 65 - protein, 17 aa, synthetic construct
  REGION 1..17: note = artificial peptide
  MUTAGEN 2: note = X stands for 1-naphthyl-L-alanine
  MUTAGEN 7: note = X stands for 3-[(aminoiminomethyl)amino]-L-phenylalanine
  MUTAGEN 10: note = X stands for phenethylglycine
  MUTAGEN 12: note = X stands for 1-naphthyl-L-alanine
FXVVNVXDDXVXYHVCG

SEQ ID NO: 66 - protein, 17 aa, synthetic construct
  REGION 1..17: note = artificial peptide
  MUTAGEN 2: note = X stands for L-7-azatryptophan
  MUTAGEN 10: note = X stands for phenethylglycine
  MUTAGEN 12: note = X stands for 1-naphthyl-L-alanine
FXVVNVYDDXVXYHVCG

SEQ ID NO: 67 - protein, 17 aa, synthetic construct
  REGION 1..17: note = artificial peptide
  MUTAGEN 2: note = X stands for 1-naphthyl-L-alanine
  MUTAGEN 10: note = X stands for phenethylglycine
  MUTAGEN 12: note = X stands for 1-naphthyl-L-alanine
FXVVNVYDEXVXYHVCG

SEQ ID NO: 68 - protein, 17 aa, synthetic construct
  REGION 1..17: note = artificial peptide
  MUTAGEN 2: note = X stands for 1-naphthyl-L-alanine
  MUTAGEN 7: note = X stands for 4-pyridyl-L-alanine
  MUTAGEN 10: note = X stands for phenethylglycine
  MUTAGEN 12: note = X stands for 1-naphthyl-L-alanine
FXVVNVXDDXVXYHVCG

SEQ ID NO: 69 - protein, 17 aa, synthetic construct
  REGION 1..17: note = artificial peptide
  MUTAGEN 2: note = X stands for 1-naphthyl-L-alanine
  MUTAGEN 7: note = X stands for 3-(3-pyridyl)-L-alanine
  MUTAGEN 10: note = X stands for phenethylglycine
  MUTAGEN 12: note = X stands for 1-naphthyl-L-alanine
FXVVNVXDDXVXYHVCG

SEQ ID NO: 70 - protein, 9 aa, synthetic construct
  REGION 1..9: note = artificial peptide
  BINDING 1: note = Tyr is bouded by 1-amino-3, 6, 9, 12, 15, 18, 21, 24, 27, 30-decaoxatritriacontane-33-oic acid
YPYDVPDYA